European Patent Application EP 4 527 853 A1, published March 26, 2025. Title: PD-L1 및 CD47에 대한 이중특이적 인간화 단일 도메인 항체 및 이의 용도. Applicant: (주)샤페론. Application KR. The sequence listing filed with the application follows.

SEQUENCE LISTING (32 sequences)

SEQ ID NO: 1 - protein, 120 aa, synthetic construct
  REGION 1..120: note = PDL1 Nb#01
QVQLVESGGGLVQPGGSLRLSCAASGFTFSSFAMSWVRQAPGKGLEWVSDINTGGDSTDYADSVKGRFTISRDNAKNTLYLQMNSLKPEDTAVYYCAKGPKEMVHVYSQRGQGTQVTVSS

SEQ ID NO: 2 - protein, 8 aa, synthetic construct
  REGION 1..8: note = PDL1 Nb#01_CDR1
GFTFSSFA

SEQ ID NO: 3 - protein, 8 aa, synthetic construct
  REGION 1..8: note = PDL1 Nb#01_CDR2
INTGGDST

SEQ ID NO: 4 - protein, 13 aa, synthetic construct
  REGION 1..13: note = PDL1 Nb#01_CDR3
AKGPKEMVHVYSQ

SEQ ID NO: 5 - protein, 357 aa, synthetic construct
  REGION 1..357: note = PDL1 Nb#01-IgG1
QVQLVESGGGLVQPGGSLRLSCAASGFTFSSFAMSWVRQAPGKGLEWVSDINTGGDSTDYADSVKGRFTISRDNAKNTLYLQMNSLKPEDTAVYYCAKGPKEMVHVYSQRGQGTQVTVSSGPGGPEPKSSDKTHTCPPCPAPELLGGPSVFLFPPKPKDTLMISRTPEVTCVVVDVSHEDPEVKFNWYVDGVEVHNAKTKPREEQYNSTYRVVSVLTVLHQDWLNGKEYKCKVSNKALPAPIEKTISKAKGQPREPQVYTLPPSRDELTKNQVSLTCLVKGFYPSDIAVEWESNGQPENNYKTTPPVLDSDGSFFLYSKLTVDKSRWQQGNVFSCSVMHEALHNHYTQKSLSLSPGK

SEQ ID NO: 6 - protein, 246 aa, synthetic construct
  REGION 1..246: note = PP Nb
QVQLVESGGGLVQPGGSLRLSCAASGFTFSSFAMSWVRQAPGKGLEWVSDINTGGDSTDYADSVKGRFTISRDNAKNTLYLQMNSLKPEDTAVYYCAKGPKEMVHVYSQRGQGTQVTVSSGGSGGSQVQLVESGGGLVQPGGSLRLSCAASGFTFSSFAMSWVRQAPGKGLEWVSDINTGGDSTDYADSVKGRFTISRDNAKNTLYLQMNSLKPEDTAVYYCAKGPKEMVHVYSQRGQGTQVTVSS

SEQ ID NO: 7 - protein, 480 aa, synthetic construct
  REGION 1..480: note = PP Nb-IgG4
QVQLVESGGGLVQPGGSLRLSCAASGFTFSSFAMSWVRQAPGKGLEWVSDINTGGDSTDYADSVKGRFTISRDNAKNTLYLQMNSLKPEDTAVYYCAKGPKEMVHVYSQRGQGTQVTVSSGGSGGSQVQLVESGGGLVQPGGSLRLSCAASGFTFSSFAMSWVRQAPGKGLEWVSDINTGGDSTDYADSVKGRFTISRDNAKNTLYLQMNSLKPEDTAVYYCAKGPKEMVHVYSQRGQGTQVTVSSGPGGPESKYGPPCPPCPAPEFLGGPSVFLFPPKPKDTLMISRTPEVTCVVVDVSQEDPEVQFNWYVDGVEVHNAKTKPREEQFNSTYRVVSVLTVLHQDWLNGKEYKCKVSNKGLPSSIEKTISKAKGQPREPQVYTLPPSQEEMTKNQVSLTCLVKGFYPSDIAVEWESNGQPENNYKTTPPVLDSDGSFFLYSRLTVDKSRWQEGNVFSCSVMHEALHNHYTQKSLSLSPGK

SEQ ID NO: 8 - protein, 123 aa, synthetic construct
  REGION 1..123: note = CD47 Nb#01
QVQLVESGGGLVQPGGSLNLSCAVSGLTFFRKYAVGWARQVPGKGLERVSRIYSDRRIEYLDAVKGRFTISRDNAKNTVYLQMNSLKTEDTAVYYCATGLRVGLTGWDEYDYWGQGTQVTVSS

SEQ ID NO: 9 - protein, 9 aa, synthetic construct
  REGION 1..9: note = CD47 Nb#01_CDR1
GLTFFRKYA

SEQ ID NO: 10 - protein, 7 aa, synthetic construct
  REGION 1..7: note = CD47 Nb#01_CDR2
IYSDRRI

SEQ ID NO: 11 - protein, 16 aa, synthetic construct
  REGION 1..16: note = CD47 Nb#01_CDR3
ATGLRVGLTGWDEYDY

SEQ ID NO: 12 - protein, 357 aa, synthetic construct
  REGION 1..357: note = CD47 Nb-IgG4
QVQLVESGGGLVQPGGSLNLSCAVSGLTFFRKYAVGWARQVPGKGLERVSRIYSDRRIEYLDAVKGRFTISRDNAKNTVYLQMNSLKTEDTAVYYCATGLRVGLTGWDEYDYWGQGTQVTVSSGPGGPESKYGPPCPPCPAPEFLGGPSVFLFPPKPKDTLMISRTPEVTCVVVDVSQEDPEVQFNWYVDGVEVHNAKTKPREEQFNSTYRVVSVLTVLHQDWLNGKEYKCKVSNKGLPSSIEKTISKAKGQPREPQVYTLPPSQEEMTKNQVSLTCLVKGFYPSDIAVEWESNGQPENNYKTTPPVLDSDGSFFLYSRLTVDKSRWQEGNVFSCSVMHEALHNHYTQKSLSLSPGK

SEQ ID NO: 13 - protein, 380 aa, synthetic construct
  REGION 1..380: note = PPC Nb
QVQLVESGGGLVQPGGSLRLSCAASGFTFSSFAMSWVRQAPGKGLEWVSDINTGGDSTDYADSVKGRFTISRDNAKNTLYLQMNSLKPEDTAVYYCAKGPKEMVHVYSQRGQGTQVTVSSGGSGGGPSQVQLVESGGGLVQPGGSLRLSCAASGFTFSSFAMSWVRQAPGKGLEWVSDINTGGDSTDYADSVKGRFTISRDNAKNTLYLQMNSLKPEDTAVYYCAKGPKEMVHVYSQRGQGTQVTVSSGGSGGSGGSQVQLVESGGGLVQPGGSLNLSCAVSGLTFFRKYAVGWARQVPGKGLERVSRIYSDRRIEYLDAVKGRFTISRDNAKNTVYLQMNSLKTEDTAVYYCATGLRVGLTGWDEYDYWGQGTQVTVSS

SEQ ID NO: 14 - protein, 614 aa, synthetic construct
  REGION 1..614: note = PPC Nb-IgG4
QVQLVESGGGLVQPGGSLRLSCAASGFTFSSFAMSWVRQAPGKGLEWVSDINTGGDSTDYADSVKGRFTISRDNAKNTLYLQMNSLKPEDTAVYYCAKGPKEMVHVYSQRGQGTQVTVSSGGSGGGPSQVQLVESGGGLVQPGGSLRLSCAASGFTFSSFAMSWVRQAPGKGLEWVSDINTGGDSTDYADSVKGRFTISRDNAKNTLYLQMNSLKPEDTAVYYCAKGPKEMVHVYSQRGQGTQVTVSSGGSGGSGGSQVQLVESGGGLVQPGGSLNLSCAVSGLTFFRKYAVGWARQVPGKGLERVSRIYSDRRIEYLDAVKGRFTISRDNAKNTVYLQMNSLKTEDTAVYYCATGLRVGLTGWDEYDYWGQGTQVTVSSGPGGPESKYGPPCPPCPAPEFLGGPSVFLFPPKPKDTLMISRTPEVTCVVVDVSQEDPEVQFNWYVDGVEVHNAKTKPREEQFNSTYRVVSVLTVLHQDWLNGKEYKCKVSNKGLPSSIEKTISKAKGQPREPQVYTLPPSQEEMTKNQVSLTCLVKGFYPSDIAVEWESNGQPENNYKTTPPVLDSDGSFFLYSRLTVDKSRWQEGNVFSCSVMHEALHNHYTQKSLSLSPGK

SEQ ID NO: 15 - protein, 380 aa, synthetic construct
  REGION 1..380: note = hPPC Nb
EVQLVESGGGLVQPGGSLRLSCAASGFTFSSFAMSWVRQAPGKGLEWVSDINTGGDSTDYADSVKGRFTISRDNAKNTLYLQMNSLKPEDTAVYYCAKGPKEMVHVYSQRGQGTQVTVSSGGSGGGPSEVQLVESGGGLVQPGGSLRLSCAASGFTFSSFAMSWVRQAPGKGLEWVSDINTGGDSTDYADSVKGRFTISRDNAKNTLYLQMNSLKPEDTAVYYCAKGPKEMVHVYSQRGQGTQVTVSSGGSGGSGGSEVQLVESGGGLVQPGGSLNLSCAVSGLTFFRKYAVGWARQVPGKGLERVSRIYSDRRIEYLDAVKGRFTISRDNAKNTVYLQMNSLKTEDTAVYYCATGLRVGLTGWDEYDYWGQGTQVTVSS

SEQ ID NO: 16 - protein, 120 aa, synthetic construct
  REGION 1..120: note = hPDL1 Nb#01
EVQLVESGGGLVQPGGSLRLSCAASGFTFSSFAMSWVRQAPGKGLEWVSDINTGGDSTDYADSVKGRFTISRDNAKNTLYLQMNSLKPEDTAVYYCAKGPKEMVHVYSQRGQGTQVTVSS

SEQ ID NO: 17 - protein, 123 aa, synthetic construct
  REGION 1..123: note = hCD47 Nb#01
EVQLVESGGGLVQPGGSLNLSCAVSGLTFFRKYAVGWARQVPGKGLERVSRIYSDRRIEYLDAVKGRFTISRDNAKNTVYLQMNSLKTEDTAVYYCATGLRVGLTGWDEYDYWGQGTQVTVSS

SEQ ID NO: 18 - protein, 614 aa, synthetic construct
  REGION 1..614: note = hPPC Nb-IgG4
EVQLVESGGGLVQPGGSLRLSCAASGFTFSSFAMSWVRQAPGKGLEWVSDINTGGDSTDYADSVKGRFTISRDNAKNTLYLQMNSLKPEDTAVYYCAKGPKEMVHVYSQRGQGTQVTVSSGGSGGGPSEVQLVESGGGLVQPGGSLRLSCAASGFTFSSFAMSWVRQAPGKGLEWVSDINTGGDSTDYADSVKGRFTISRDNAKNTLYLQMNSLKPEDTAVYYCAKGPKEMVHVYSQRGQGTQVTVSSGGSGGSGGSEVQLVESGGGLVQPGGSLNLSCAVSGLTFFRKYAVGWARQVPGKGLERVSRIYSDRRIEYLDAVKGRFTISRDNAKNTVYLQMNSLKTEDTAVYYCATGLRVGLTGWDEYDYWGQGTQVTVSSGPGGPESKYGPPCPPCPAPEFLGGPSVFLFPPKPKDTLMISRTPEVTCVVVDVSQEDPEVQFNWYVDGVEVHNAKTKPREEQFNSTYRVVSVLTVLHQDWLNGKEYKCKVSNKGLPSSIEKTISKAKGQPREPQVYTLPPSQEEMTKNQVSLTCLVKGFYPSDIAVEWESNGQPENNYKTTPPVLDSDGSFFLYSRLTVDKSRWQEGNVFSCSVMHEALHNHYTQKSLSLSPGK

SEQ ID NO: 19 - protein, 25 aa, synthetic construct [sequence omitted]

SEQ ID NO: 20 - protein, 17 aa, synthetic construct
  REGION 1..17: note = hPDL1 Nb#01_FR2
MSWVRQAPGKGLEWVSD

SEQ ID NO: 21 - protein, 38 aa, synthetic construct
  REGION 1..38: note = hPDL1 Nb#01_FR3
DYADSVKGRFTISRDNAKNTLYLQMNSLKPEDTAVYYC

SEQ ID NO: 22 - protein, 11 aa, synthetic construct
  REGION 1..11: note = hPDL1 Nb#01_FR4
RGQGTQVTVSS

SEQ ID NO: 23 - protein, 25 aa, synthetic construct
  REGION 1..25: note = hCD47 Nb#01_FR1
EVQLVESGGGLVQPGGSLNLSCAVS

SEQ ID NO: 24 - protein, 17 aa, synthetic construct
  REGION 1..17: note = hCD47 Nb#01_FR2
VGWARQVPGKGLERVSR

SEQ ID NO: 25 - protein, 38 aa, synthetic construct
  REGION 1..38: note = hCD47 Nb#01_FR3
EYLDAVKGRFTISRDNAKNTVYLQMNSLKTEDTAVYYC

SEQ ID NO: 26 - protein, 11 aa, synthetic construct
  REGION 1..11: note = hCD47 Nb#01_FR4
WGQGTQVTVSS

SEQ ID NO: 27 - protein, 6 aa, synthetic construct
  REGION 1..6: note = Peptide linker_1
GGSGGS

SEQ ID NO: 28 - protein, 8 aa, synthetic construct
  REGION 1..8: note = Peptide linker_2
GGSGGGPS

SEQ ID NO: 29 - protein, 9 aa, synthetic construct
  REGION 1..9: note = Peptide linker_3
GGSGGSGGS

SEQ ID NO: 30 - protein, 5 aa, synthetic construct
  REGION 1..5: note = Peptide linker_4
GPGGP

SEQ ID NO: 31 - protein, 482 aa, synthetic construct
  REGION 1..482: note = hPP Nb-IgG4
EVQLVESGGGLVQPGGSLRLSCAASGFTFSSFAMSWVRQAPGKGLEWVSDINTGGDSTDYADSVKGRFTISRDNAKNTLYLQMNSLKPEDTAVYYCAKGPKEMVHVYSQRGQGTQVTVSSGGSGGGPSEVQLVESGGGLVQPGGSLRLSCAASGFTFSSFAMSWVRQAPGKGLEWVSDINTGGDSTDYADSVKGRFTISRDNAKNTLYLQMNSLKPEDTAVYYCAKGPKEMVHVYSQRGQGTQVTVSSGPGGPESKYGPPCPPCPAPEFLGGPSVFLFPPKPKDTLMISRTPEVTCVVVDVSQEDPEVQFNWYVDGVEVHNAKTKPREEQFNSTYRVVSVLTVLHQDWLNGKEYKCKVSNKGLPSSIEKTISKAKGQPREPQVYTLPPSQEEMTKNQVSLTCLVKGFYPSDIAVEWESNGQPENNYKTTPPVLDSDGSFFLYSRLTVDKSRWQEGNVFSCSVMHEALHNHYTQKSLSLSPGK

SEQ ID NO: 32 - protein, 357 aa, unidentified
  REGION 1..357: note = hCD47 Nb-IgG4
EVQLVESGGGLVQPGGSLNLSCAVSGLTFFRKYAVGWARQVPGKGLERVSRIYSDRRIEYLDAVKGRFTISRDNAKNTVYLQMNSLKTEDTAVYYCATGLRVGLTGWDEYDYWGQGTQVTVSSGPGGPESKYGPPCPPCPAPEFLGGPSVFLFPPKPKDTLMISRTPEVTCVVVDVSQEDPEVQFNWYVDGVEVHNAKTKPREEQFNSTYRVVSVLTVLHQDWLNGKEYKCKVSNKGLPSSIEKTISKAKGQPREPQVYTLPPSQEEMTKNQVSLTCLVKGFYPSDIAVEWESNGQPENNYKTTPPVLDSDGSFFLYSRLTVDKSRWQEGNVFSCSVMHEALHNHYTQKSLSLSPGK